European Patent Application EP 4 631 973 A1, published October 15, 2025. Title: Novel triple GLP-1/GIP/glucagon receptor agonist and a pharmaceutical composition for preventing or treating obesity comprising the same. Applicant: HANMI PHARM. CO., LTD. The sequence listing filed with the application follows.

SEQUENCE LISTING (29 sequences)

SEQ ID NO: 1 - protein, 39 aa, synthetic construct
  SITE 2: note = X is 2-aminoisobutyric acid (Aib)
  SITE 16..20: note = Amino acids at positions 16 and 20 form a ring
  SITE 12: note = X is C20diacid-gammaGlu-(AEEA)2-Lys
YXQGTFTSDYSXYLDEKAAKEFVQWLLDHHPSSGQPPPS

SEQ ID NO: 2 - protein, 39 aa, synthetic construct
  SITE 2: note = X is 2-aminoisobutyric acid (Aib)
  SITE 16..20: note = Amino acids at positions 16 and 20 form a ring
  SITE 12: note = X is C20diacid-gammaGlu-(AEEA)2-Lys
YXQGTFTSDYSXYLDEKRAKEFVQWLLDHHPSSGQPPPS

SEQ ID NO: 3 - protein, 39 aa, synthetic construct
  SITE 2: note = X is 2-aminoisobutyric acid (Aib)
  SITE 12: note = X is C20diacid-gammaGlu-(AEEA)2-Lys
  SITE 16..20: note = Amino acids at positions 16 and 20 form a ring
YXQGTFTSDYSXYLDEKAAKDFVQWLLDQHPSSGQPPPS

SEQ ID NO: 4 - protein, 39 aa, synthetic construct
  SITE 2: note = X is 2-aminoisobutyric acid (Aib)
  SITE 12: note = X is C20diacid-gammaGlu-(AEEA)2-Lys
  SITE 16..20: note = Amino acids at positions 16 and 20 form a ring
YXQGTFTSDYSXYLDEKRAKDFVQWLLDHHPSSGQPPPS

SEQ ID NO: 5 - protein, 39 aa, synthetic construct
  SITE 2: note = X is 2-aminoisobutyric acid (Aib)
  SITE 12: note = X is C20diacid-gammaGlu-(AEEA)2-Lys
  SITE 16..20: note = Amino acids at positions 16 and 20 form a ring
YXQGTFTSDYSXALDEKRAKEFVQWLLDQHPSSGQPPPS

SEQ ID NO: 6 - protein, 39 aa, synthetic construct
  SITE 2: note = X is 2-aminoisobutyric acid (Aib)
  SITE 12: note = X is C20diacid-gammaGlu-(AEEA)2-Lys
  SITE 16..20: note = Amino acids at positions 16 and 20 form a ring
HXHGTFTSDYSXYLDEKAAKDFVQWLLDQHPSSGQPPPS

SEQ ID NO: 7 - protein, 39 aa, synthetic construct
  SITE 2: note = X is 2-aminoisobutyric acid (Aib)
  SITE 12: note = X is C20diacid-gammaGlu-(AEEA)2-Lys
  SITE 16..20: note = Amino acids at positions 16 and 20 form a ring
YXQGTFTSDYSXYLDEKRAKDFVQWLLDQHPSSGQPPPS

SEQ ID NO: 8 - protein, 39 aa, synthetic construct; identical to SEQ ID NO: 2
  SITE 2: note = X is 2-aminoisobutyric acid (Aib)
  SITE 12: note = X is C18diacid-gammaGlu-(AEEA)2-Lys
  SITE 16..20: note = Amino acids at positions 16 and 20 form a ring

SEQ ID NO: 9 - protein, 39 aa, synthetic construct; identical to SEQ ID NO: 1
  SITE 2: note = X is 2-aminoisobutyric acid (Aib)
  SITE 12: note = X is C18diacid-gammaGlu-(AEEA)2-Lys
  SITE 16..20: note = Amino acids at positions 16 and 20 form a ring

SEQ ID NO: 10 - protein, 39 aa, synthetic construct; identical to SEQ ID NO: 3
  SITE 12: note = X is C18diacid-gammaGlu-(AEEA)2-Lys
  SITE 2: note = X is 2-aminoisobutyric acid (Aib)
  SITE 16..20: note = Amino acids at positions 16 and 20 form a ring

SEQ ID NO: 11 - protein, 39 aa, synthetic construct; identical to SEQ ID NO: 4
  SITE 2: note = X is 2-aminoisobutyric acid (Aib)
  SITE 12: note = X is C18diacid-gammaGlu-(AEEA)2-Lys
  SITE 16..20: note = Amino acids at positions 16 and 20 form a ring

SEQ ID NO: 12 - protein, 39 aa, synthetic construct; identical to SEQ ID NO: 5
  SITE 2: note = X is 2-aminoisobutyric acid (Aib)
  SITE 12: note = X is C18diacid-gammaGlu-(AEEA)2-Lys
  SITE 16..20: note = Amino acids at positions 16 and 20 form a ring

SEQ ID NO: 13 - protein, 39 aa, synthetic construct; identical to SEQ ID NO: 6
  SITE 2: note = X is 2-aminoisobutyric acid (Aib)
  SITE 12: note = X is C18diacid-gammaGlu-(AEEA)2-Lys
  SITE 16..20: note = Amino acids at positions 16 and 20 form a ring

SEQ ID NO: 14 - protein, 39 aa, synthetic construct; identical to SEQ ID NO: 7
  SITE 2: note = X is 2-aminoisobutyric acid (Aib)
  SITE 12: note = X is C18diacid-gammaGlu-(AEEA)2-Lys
  SITE 16..20: note = Amino acids at positions 16 and 20 form a ring

SEQ ID NO: 15 - protein, 39 aa, synthetic construct
  SITE 2: note = X is 2-aminoisobutyric acid (Aib)
  SITE 17: note = X is C20diacid-gammaGlu-(AEEA)2-Lys
  SITE 16..20: note = Amino acids at positions 16 and 20 form a ring
YXQGTFTSDYSKYLDEXAAKEFVQWLLDHHPSSGQPPPS

SEQ ID NO: 16 - protein, 39 aa, synthetic construct
  SITE 2: note = X is 2-aminoisobutyric acid (Aib)
  SITE 17: note = X is C20diacid-gammaGlu-(AEEA)2-Lys
  SITE 16..20: note = Amino acids at positions 16 and 20 form a ring
YXQGTFTSDYSKYLDEXRAKEFVQWLLDHHPSSGQPPPS

SEQ ID NO: 17 - protein, 39 aa, synthetic construct
  SITE 2: note = X is 2-aminoisobutyric acid (Aib)
  SITE 17: note = X is C20diacid-gammaGlu-(AEEA)2-Lys
  SITE 16..20: note = Amino acids at positions 16 and 20 form a ring
YXQGTFTSDYSKYLDEXAAKDFVQWLLDQHPSSGQPPPS

SEQ ID NO: 18 - protein, 39 aa, synthetic construct
  SITE 2: note = X is 2-aminoisobutyric acid (Aib)
  SITE 17: note = X is C20diacid-gammaGlu-(AEEA)2-Lys
  SITE 16..20: note = Amino acids at positions 16 and 20 form a ring
YXQGTFTSDYSKYLDEXRAKDFVQWLLDHHPSSGQPPPS

SEQ ID NO: 19 - protein, 39 aa, synthetic construct
  SITE 2: note = X is 2-aminoisobutyric acid (Aib)
  SITE 17: note = X is C20diacid-gammaGlu-(AEEA)2-Lys
  SITE 16..20: note = Amino acids at positions 16 and 20 form a ring
YXQGTFTSDYSKALDEXRAKEFVQWLLDQHPSSGQPPPS

SEQ ID NO: 20 - protein, 39 aa, synthetic construct
  SITE 17: note = X is C20diacid-gammaGlu-(AEEA)2-Lys
  SITE 2: note = X is 2-aminoisobutyric acid (Aib)
  SITE 16..20: note = Amino acids at positions 16 and 20 form a ring
HXHGTFTSDYSKYLDEXAAKDFVQWLLDQHPSSGQPPPS

SEQ ID NO: 21 - protein, 39 aa, synthetic construct
  SITE 2: note = X is 2-aminoisobutyric acid (Aib)
  SITE 17: note = X is C20diacid-gammaGlu-(AEEA)2-Lys
  SITE 16..20: note = Amino acids at positions 16 and 20 form a ring
YXQGTFTSDYSKYLDEXRAKDFVQWLLDQHPSSGQPPPS

SEQ ID NO: 22 - protein, 39 aa, synthetic construct; identical to SEQ ID NO: 15
  SITE 17: note = X is C18diacid-gammaGlu-(AEEA)2-Lys
  SITE 2: note = X is 2-aminoisobutyric acid (Aib)
  SITE 16..20: note = Amino acids at positions 16 and 20 form a ring

SEQ ID NO: 23 - protein, 39 aa, synthetic construct; identical to SEQ ID NO: 16
  SITE 17: note = X is C18diacid-gammaGlu-(AEEA)2-Lys
  SITE 2: note = X is 2-aminoisobutyric acid (Aib)
  SITE 16..20: note = Amino acids at positions 16 and 20 form a ring

SEQ ID NO: 24 - protein, 39 aa, synthetic construct; identical to SEQ ID NO: 17
  SITE 2: note = X is 2-aminoisobutyric acid (Aib)
  SITE 17: note = X is C18diacid-gammaGlu-(AEEA)2-Lys
  SITE 16..20: note = Amino acids at positions 16 and 20 form a ring

SEQ ID NO: 25 - protein, 39 aa, synthetic construct; identical to SEQ ID NO: 18
  SITE 2: note = X is 2-aminoisobutyric acid (Aib)
  SITE 17: note = X is C18diacid-gammaGlu-(AEEA)2-Lys
  SITE 16..20: note = Amino acids at positions 16 and 20 form a ring

SEQ ID NO: 26 - protein, 39 aa, synthetic construct; identical to SEQ ID NO: 19
  SITE 2: note = X is 2-aminoisobutyric acid (Aib)
  SITE 17: note = X is C18diacid-gammaGlu-(AEEA)2-Lys
  SITE 16..20: note = Amino acids at positions 16 and 20 form a ring

SEQ ID NO: 27 - protein, 39 aa, synthetic construct; identical to SEQ ID NO: 20
  SITE 17: note = X is C18diacid-gammaGlu-(AEEA)2-Lys
  SITE 2: note = X is 2-aminoisobutyric acid (Aib)
  SITE 16..20: note = Amino acids at positions 16 and 20 form a ring

SEQ ID NO: 28 - protein, 39 aa, synthetic construct; identical to SEQ ID NO: 21
  SITE 2: note = X is 2-aminoisobutyric acid (Aib)
  SITE 17: note = X is C18diacid-gammaGlu-(AEEA)2-Lys
  SITE 16..20: note = Amino acids at positions 16 and 20 form a ring

SEQ ID NO: 29 - protein, 39 aa, synthetic construct
  SITE 1: note = X is histidine or tyrosine
  SITE 2: note = X is 2-aminoisobutyric acid (Aib)
  SITE 3: note = X is glutamine or histidine
  SITE 12: note = X is lysine or acylated amino acid
  SITE 13: note = X is alpha-methyl-leucine, tyrosine or alanine
  SITE 18: note = X is alanine or arginine
  SITE 17: note = X is lysine or acylated amino acid
  SITE 21: note = X is aspartic acid or glutamic acid
  SITE 29: note = X is histidine or glutamine
XXXGTFTSDYSXXLDEXXAKXFVQWLLDXHPSSGQPPPS